European Patent Application EP 4 151 739 A1, published March 22, 2023. Title: IMPROVED TRANSPOSON SYSTEM FOR GENE DELIVERY. Applicant: T-CURX GmbH. Application EP. The sequence listing filed with the application follows.

SEQUENCE LISTING (19 sequences)

SEQ ID NO: 1 - protein, 340 aa, synthetic construct
  REGION 1..340: note = hyperactive SB transposase SB100X
MGKSKEISQDLRKRIVDLHKSGSSLGAISKRLAVPRSSVQTIVRKYKHHGTTQPSYRSGRRRVLSPRDERTLVRKVQINPRTTAKDLVKMLEETGTKVSISTVKRVLYRHNLKGHSARKKPLLQNRHKKARLRFATAHGDKDRTFWRNVLWSDETKIELFGHNDHRYVWRKKGEACKPKNTIPTVKHGGGSIMLWGCFAAGGTGALHKIDGIMDAVQYVDILKQHLKTSVRKLKLGRKWVFQHDNDPKHTSKVVAKWLKDNKVKVLEWPSQSPDLNPIENLWAELKKRVRARRPTNLTQLHQLCQEEWAKIHPNYCGKLVEGYPKRLTQVKQFKGNATKY

SEQ ID NO: 2 - RNA, 1218 nt, synthetic construct
  misc_feature 1..1218: note = Sequence of SB100XmCo SNIM RNA resulting from in-vitrotranscription from pVAXA120-SB100XmCo
  source 1..1218: mol_type = other RNA
gggagacccaagctggctagcgtttaaacttaagcttggtaccgagctcggatccaccatgggcaagagcaaagagatcagccaggacctgagaaagcggatcgtggacctgcacaagagcggctctagcctgggcgccatcagcaagagactggccgtgcctagaagcagcgtgcagaccatcgtgcggaagtacaagcaccacggcaccacccagcccagctacagatctgggagaagaagagtgctgagccccagggacgagagaaccctcgtgcgcaaggtgcagatcaaccccagaaccaccgccaaggacctcgtgaagatgctggaagagacaggcaccaaggtgtccatcagcaccgtgaagagggtgctgtacagacacaacctgaagggccacagcgccagaaagaagcccctgctgcagaacaggcacaagaaggccagactgagattcgccaccgcccacggcgacaaggacagaaccttttggagaaacgtgctgtggagcgacgagacaaagatcgagctgttcggccacaacgaccacagatacgtgtggcggaagaagggcgaggcctgcaagcccaagaacaccatccctaccgtgaagcacggcggaggcagcatcatgctgtggggctgttttgccgctggcggcacaggcgccctgcataagatcgacggcatcatggacgccgtgcagtacgtggacatcctgaagcagcacctgaaaacctctgtgcggaagctgaagctgggcagaaaatgggtgttccagcacgacaacgaccccaagcacaccagcaaggtggtggccaagtggctgaaggacaacaaagtgaaagtgctggaatggcccagccagagccccgacctgaaccccatcgagaacctgtgggccgagctgaagaaaagagtgcgggccagaaggcccaccaacctgacacagctgcaccagctgtgccaggaagagtgggccaagatccaccccaactactgcggcaagctggtggaaggctaccccaagaggctgacccaagtgaagcagttcaagggcaacgccaccaagtactgagaattctgcagaaaaaaaaaaaaaaaaaaaaaaaaaaaaaaaaaaaaaaaaaaaaaaaaaaaaaaaaaaaaaaaaaaaaaaaaaaaaaaaaaaaaaaaaaaaaaaaaaaaaaaaaaaaaaaaaaaaaaaaagcggcc

SEQ ID NO: 3 - RNA, 1218 nt, synthetic construct
  misc_feature 1..1218: note = Sequence of SB100XmCo(DAE) SNIM RNA resulting from in-vitrotranscription from pVAXA120-SB100XmCo(DAE)
  source 1..1218: mol_type = other RNA
gggagacccaagctggctagcgtttaaacttaagcttggtaccgagctcggatccaccatgggcaagagcaaagagatcagccaggacctgagaaagcggatcgtggacctgcacaagagcggctctagcctgggcgccatcagcaagagactggccgtgcctagaagcagcgtgcagaccatcgtgcggaagtacaagcaccacggcaccacccagcccagctacagatctgggagaagaagagtgctgagccccagggacgagagaaccctcgtgcgcaaggtgcagatcaaccccagaaccaccgccaaggacctcgtgaagatgctggaagagacaggcaccaaggtgtccatcagcaccgtgaagagggtgctgtacagacacaacctgaagggccacagcgccagaaagaagcccctgctgcagaacaggcacaagaaggccagactgagattcgccaccgcccacggcgacaaggacagaaccttttggagaaacgtgctgtggagcgacgagacaaagatcgagctgttcggccacaacgaccacagatacgtgtggcggaagaagggcgaggcctgcaagcccaagaacaccatccctaccgtgaagcacggcggaggcagcatcatgctgtggggctgttttgccgctggcggcacaggcgccctgcataagatcgacggcatcatggacgccgtgcagtacgtggacatcctgaagcagcacctgaaaacctctgtgcggaagctgaagctgggcagaaaatgggtgttccagcacgccaacgaccccaagcacaccagcaaggtggtggccaagtggctgaaggacaacaaagtgaaagtgctggaatggcccagccagagccccgacctgaaccccatcgagaacctgtgggccgagctgaagaaaagagtgcgggccagaaggcccaccaacctgacacagctgcaccagctgtgccaggaagagtgggccaagatccaccccaactactgcggcaagctggtggaaggctaccccaagaggctgacccaagtgaagcagttcaagggcaacgccaccaagtactgagaattctgcagaaaaaaaaaaaaaaaaaaaaaaaaaaaaaaaaaaaaaaaaaaaaaaaaaaaaaaaaaaaaaaaaaaaaaaaaaaaaaaaaaaaaaaaaaaaaaaaaaaaaaaaaaaaaaaaaaaaaaaaagcggcc

SEQ ID NO: 4 - DNA, 34 bp, synthetic construct
  misc_feature 1..34: note = ITR of the transposon unit termed Lo
  source 1..34: mol_type = other DNA
tacagttgaagtcggaagtttacatacacttaag

SEQ ID NO: 5 - DNA, 32 bp, synthetic construct
  misc_feature 1..32: note = ITR of the transposon unit termed Li
  source 1..32: mol_type = other DNA
tccagtgggtcagaagtttacatacactaagt

SEQ ID NO: 6 - DNA, 32 bp, synthetic construct
  misc_feature 1..32: note = ITR of the transposon unit termed Ri
  source 1..32: mol_type = other DNA
cccagtgggtcagaagtttacatacactcaat

SEQ ID NO: 7 - DNA, 34 bp, synthetic construct
  misc_feature 1..34: note = ITR of the transposon unit termed Ro
  source 1..34: mol_type = other DNA
tacagttgaagtcggaagtttacatacaccttag

SEQ ID NO: 8 - DNA, 34 bp, synthetic construct
  misc_feature 1..34: note = ITR of the transposon unit termed DRo
  source 1..34: mol_type = other DNA
tacagttgaagtcggaagtttacatacacytaag

SEQ ID NO: 9 - DNA, 30 bp, synthetic construct
  misc_feature 1..30: note = ITR of the transposon unit termed DRi
  source 1..30: mol_type = other DNA
cagtgggtcagaagtttacatacactmart

SEQ ID NO: 10 - DNA, 35 bp, synthetic construct
  misc_feature 1..35: note = Primer SB-IRDR-R_FW
  source 1..35: mol_type = other DNA
gctgaaatgaatcattctctctactattattctga

SEQ ID NO: 11 - DNA, 26 bp, synthetic construct
  misc_feature 1..26: note = Primer SB-IRDR-R_RV
  source 1..26: mol_type = other DNA
aattccctgtcttaggtcagttagga

SEQ ID NO: 12 - DNA, 20 bp, synthetic construct
  misc_feature 1..20: note = Primer TERT_FW
  source 1..20: mol_type = other DNA
gacaaagtacagctcaggcg

SEQ ID NO: 13 - DNA, 20 bp, synthetic construct
  misc_feature 1..20: note = Primer TERT_RV
  source 1..20: mol_type = other DNA
ttcagcgtgctcaactacga

SEQ ID NO: 14 - DNA, 21 bp, synthetic construct
  misc_feature 1..21: note = Primer RIR_FW
  source 1..21: mol_type = other DNA
gaatgtgatgaaagaaataaa

SEQ ID NO: 15 - DNA, 20 bp, synthetic construct
  misc_feature 1..20: note = Primer RIR_RV
  source 1..20: mol_type = other DNA
agtttacatacaccttagcc

SEQ ID NO: 16 - DNA, 27 bp, synthetic construct
  misc_feature 1..27: note = RIR-specific probe
  source 1..27: mol_type = other DNA
tggtgatcctaactgacctaagacagg

SEQ ID NO: 17 - DNA, 20 bp, synthetic construct
  misc_feature 1..20: note = Primer RPP30_FW
  source 1..20: mol_type = other DNA
ggttaactacagctcccagc

SEQ ID NO: 18 - DNA, 18 bp, synthetic construct
  misc_feature 1..18: note = Primer RPP30_RV
  source 1..18: mol_type = other DNA
ctgtctccacaagtccgc

SEQ ID NO: 19 - DNA, 24 bp, synthetic construct
  misc_feature 1..24: note = RPP30-specific probe
  source 1..24: mol_type = other DNA
tggacctgcgagcgggttctgacc